European Patent Specification EP 3 675 623 B1, published July 9, 2025. Title: IMPROVED BLUE ALEURONE AND OTHER SEGREGATION SYSTEMS. Applicant: KWS SAAT SE GLOBAL CROP INNOVATIONS PTY. LTD. THE UNIVERSITY OF SYDNEY. The sequence listing filed with the application follows.

SEQUENCE LISTING (45 sequences)

SEQ ID NO: 1 - DNA, 3838 bp, Hordeum vulgare
cgcacatcaacataaactcatcagatgggaataatcggatctacgaaggacataaaactctttaatctcatgacaacgccagaagagcaagagtaaatatattctcataaaaaacaatgaacactagatgatgacgaagaacataagattcttcaaggagaaattgcggcagcggagatggcagccggaggcgagggggccaaaaactctgttgcggcggcagcggtagccttggtgaaacccacacgtttgcacaccatataagttgtttgcaagggttacatgggcctcgctctcgtgaaaaagaaggtcatacatgggtcttggtctcgtgcaaaacgaaaggtcagcagtccatgggccggaggaaaaaccgggcaacaacacgccatgtgtgttttcgcgggaacccaattccgaaatcactcaccggcacctcgtcccgatgccttccagaacgttctacgtgcttccacagggccagcccagccgtgggatcagatcaggatcagcacgaacattgaagctagcgcggcgatatttttcccagcctccgcctcgctcgacgactgcatttcatttcgaaaacaaaaaaaagagctttctccttctcatcccgagcgccagaggagcaccagaaaggccacccacccaccctcacgtaccgccctcgcacccgcgcggccacatctgggccgtccacttgggcagctggccgttccattcccgaactgacgggcaggatcgagcgagcggcgcgcccacggctcctccggctatataacccgccacccacaccactcccctccggcgttccaccagagccttcctccctccaccgcaccaccaccaccaccgcgccaaaaaccctagggagcgagcgagctcacctcgccccgcccatggagagatcccgccgcctgctgctcgtggcggggctcctcgccgcgctgctcccggcggcggccgccaccttcgggctgcagcagggggcgcagtgcgaccccacgttcctggcgacgcaggccgcgctcttctgcgcccccgacatgcccacggcccagtgctgcgagcccgtcgtcgccgccttcgacctcgggggcggcgtcccctgcctctgccgcgtcgccgccgagccgcagctggtcatggcggggctcaacgccacccacctcttcgcgctgtacacctcctgcggcggcatccgtcccggtggcgcccacctcgccgccgcctgccaaggtacgttcacgttcaccgcctccctccctctccttctctctttgcacctgtaccagccgattcggcgttcgctttcgcgtttcccggtagttttgatggtttctcgagtcgccagtgctccgatttgggttcggtttccttgcgttgtaccggatctgcctgtacggcgcgcggcgtcggggttctcgttgtttcccgtggcgagcatccccgcgcgcccacggcctagctagcttaccttcagatacgcggagcgatttaggatcagtatgaggagttcgtcgtagaagaatgcatgcggaacgcgcgattgtttgtttcatcgattttggatctgtgataggcctgcttgttcccgagtttttgcacgtagaagaatcatgtgcagaacccctggtccattatttgttatgtatatacacgattacttgtgcatatgcagaagtcttagttatctgctacccttccagaattattcgtggtgtttttgttcctctagttaaacttcagatgatctttcgttcgagtttattttcctgcctgtaactgagatcgatatacctatcaccgtgactgtgagagagacagagagttgttgccgtttaactgctatatatatgtacgttttctgctactgtttaatcgactgctccatcccgttcgcgataggacttgtttcaaaccgtcacgcagctctgcttcctgcagtgtcttttgtcttcgtttggtcaaaactgaaaacgcttgctatcgaggccagaggcagggcaaaagctccccgtacttttcgctttgcagtggcatctctttctttttttttgccgaaaattgtttccacgttcatccccgggtgtcgtactacttaattatctgcatgcagttttcgtgtccttcctccgtcgtgaaaaaaaggttgggtcaaatgaatcaaccgtgtatgcagggcagcagcaacagagatagagtagctggctgtcgcagctttaacaaaagcagtctgtggcctgccacagttttcctgatttttgtttaatctggcctgggcttcttttcttgttgcgcacgtcgtcgcctccttcttttttcccaattttttgatttcttttgagataaggacacgaacggctggtaactgacttttcttgttgttttttactgtgggttttggacgcaggaccggctcccccggccgccgtcgtcagcagccccccgccaccatcgccagcacctcgccgcaaacaggcagcgcgtacgaacctctcgctctctctctctccctctcgcctgcatctcgctctgtacataacctattgggttcatatgctgatcagcgttgacatactaacttgttcatttgattctcagacgacgcgcctccaccgccgccgtccagcgagaagccatccccgccgccccaggagcatgacggcgccgcacacgccaagagcgcccccgccctcgcggctcctaccccgctcgcgcccgctgccgctactgccccgccgcccgaggcgccacactccgccgcgtcgtcgtccgattcggccttcatcttcatcgccgcggccatgctcgccatttacatcgtcctctgaatggccgacccccaaggcagcagagtacttgtcatctgattccgtttcatgcttgtcgccgtttgttgaggttcgtttctgcagtccgaacaagacggtggggttttgatcgggtacccagatttctatgtcgatcgcgcgtactagtactagtagttgcttagcagatgaacgaacattgggttttgggattcctctagctgatgaaccactgctattttccatgtgatcgatggatatgatctgaatggatggatgaagttttggtttctgatgctgatgatgtgctgcttcttcatttgcatgctcgatctattccttcaattttgtggagcaacagtttgtttagcttctgttctgctatgaataatgccgcttgcatcttgtcattgctgataatctgcttaatgcagacattgcttccgtcccaaacaatctgttgcttaccaggtaatgcatataatctgtacctcaccttcgcacaacaacagaagctaccctgctaaaaaaacacacacacacacacaaaaaaaacagaagctggtctcacacggaagccgcttcggggactgtttgcagctttttattgccattttgtttttcatgcaggtacaaatcgagggtgttgcttgatttgatcatggatgatcacttagagcaacatgtgtgttttgtctgtgttttattcgttgctcgtccatccaatttaaacttgaaatggatcgtgtgtggataaaagaagacgtgcgtcagtttgaatcgacgcgttgggttatattttgtgtctgtgacgaccgaaacgaagacaaaatatatcgtccggttagaattgctctaatgctagctttctctcctaccatcgcattccgtggtaggaaaaagtactagaaccacaggaaactggaacgcaagaaaagcatatctaccgttggccgttgatcttgtttcacattcggtatggctccggtcatattgttggagattcacattcatgcacgcaa

SEQ ID NO: 2 - DNA, 645 bp, Artificial Sequence
  cDNA of HvMs1
atggagagatcccgccgcctgctgctcgtggcggggctcctcgccgcgctgctcccggcggcggccgccaccttcgggctgcagcagggggcgcagtgcgaccccacgttcctggcgacgcaggccgcgctcttctgcgcccccgacatgcccacggcccagtgctgcgagcccgtcgtcgccgccttcgacctcgggggcggcgtcccctgcctctgccgcgtcgccgccgagccgcagctggtcatggcggggctcaacgccacccacctcttcgcgctgtacacctcctgcggcggcatccgtcccggtggcgcccacctcgccgccgcctgccaaggaccggctcccccggccgccgtcgtcagcagccccccgccaccatcgccagcacctcgccgcaaacaggcagcgcacgacgcgcctccaccgccgccgtccagcgagaagccatccccgccgccccaggagcatgacggcgccgcacacgccaagagcgcccccgccctcgcggctcctaccccgctcgcgcccgctgccgctactgccccgccgcccgaggcgccacactccgccgcgtcgtcgtccgattcggccttcatcttcatcgccgcggccatgctcgccatttacatcgtcctctga

SEQ ID NO: 3 - protein, 214 aa, Hordeum vulgare
MERSRRLLLVAGLLAALLPAAAATFGLQQGAQCDPTFLATQAALFCAPDMPTAQCCEPVVAAFDLGGGVPCLCRVAAEPQLVMAGLNATHLFALYTSCGGIRPGGAHLAAACQGPAPPAAVVSSPPPPSPAPRRKQAAHDAPPPPPSSEKPSPPPQEHDGAAHAKSAPALAAPTPLAPAAATAPPPEAPHSAASSSDSAFIFIAAAMLAIYIVL

SEQ ID NO: 4 - DNA, 663 bp, Artificial Sequence
  cDNA of TaMs1
atggagagatcccgcgggctgctgctggtggcggggctgctggcggcgctgctgccggcggcggcggcgcagccgggggcgccgtgcgagcccgcgctgctggcgacgcaggtggcgctcttctgcgcgcccgacatgccgacggcccagtgctgcgagcccgtcgtcgccgccgtcgacctcggcggcggggtgccctgcctctgccgcgtcgccgccgagccgcagctcgtcatggcgggcctcaacgccacccacctcctcacgctctacagctcctgcggcggcctccgccccggcggcgcccacctcgccgccgcctgcgaaggacccgctcccccggccgccgtcgtcagcagccccccgcccccgcctccaccgtccgccgcacctcgccgcaagcagccagcgcacgacgcaccaccgccgccaccgccgtcgagcgagaagccgtcgtccccgccgccgtcccaggaccacgacggcgccgccccccgcgccaaggccgcgcccgcccaggcggccacctccacgctcgcgcccgccgccgccgccaccgccccgccgccccaggcgccgcactccgccgcgcccacggcgccgtccaaggcggccttcttcttcgtcgccacggccatgctcggcctctacatcatcctctga

SEQ ID NO: 5 - protein, 220 aa, Triticum aestivum
MERSRGLLLVAGLLAALLPAAAAQPGAPCEPALLATQVALFCAPDMPTAQCCEPVVAAVDLGGGVPCLCRVAAEPQLVMAGLNATHLLTLYSSCGGLRPGGAHLAAACEGPAPPAAVVSSPPPPPPPSAAPRRKQPAHDAPPPPPPSSEKPSSPPPSQDHDGAAPRAKAAPAQAATSTLAPAAAATAPPPQAPHSAAPTAPSKAAFFFVATAMLGLYIIL

SEQ ID NO: 6 - DNA, 4335 bp, Triticum aestivum
agacttaaaccatttagttacaaatatcgatgcacaccttcggtggggcgttgtgaaaaagcatgttttttgggtcgacaagccccttttgcaacgtatcctcttctaatcctattcagatcattaacatcataagctgcaattgacatgctcttctgaggatcaggttcatgcaattaaacatcataaactgcatctttgatgtcatccttttcctatattttttccagattattggcttgcttcgttttcaatatcaggttctatgattcgacttctgttgttgccagtaataatttgtagttgctgcggaatatgaactcaaggagagctgatggtgctatgaagttgatttgatgggaggttgttctacacctgcacttgctgctcgacttaaatacatgccttggatttcttcccagctctagtacataatatttttcaaattaatgttccacgacataaaatttaaatccacaaacatatttttagtacatgaacaattttctaatatagggcaaacatttttcatatacaaaccgatcattttaatatatggtgaaaatcagtgtaatatatgctgaaatgttttcaaatacatattgaacatatttataataaatggtgaacattttttttaataattgatgaccatttttaaaatgcatattgaacattttataatatacactgtacagttttataataatcgacgaacatcttttggagttctgaacatttttttcaaaaacacaagccattttccaggaagaatacaaatgcaaaagaaatgagatatccaaaaagcaaaaaagaaaaacaaaacaaaacagagaaacctacaggaaaatccaaacagaaaaggcaaagaaagaacccgaactgggccaggcaatgtttccaacggcctcgctcttcctgaacaagaaggccagtcagcccatgggctgctcccagtactcgggccccgctgtggcagcacgccatgtaatagttttcgcgggaatccaacgccgaaatcgcccgcagcgggaacccgacgtcggtctggtgcgttctggcgccttccagaactctccacaggctcccgcagccgtccgatcagatcagcacgaagcacgaacattggcgcgcggcgatattttctttcctcgcccgacgacggccgcactgcatttcattttgaatttcaaaattcggaaacggaaaagctttctcgcatcccgaggcgaggcggttacgggcgccagaggggccaccccacccacccacccccgccctcacgtgccccgcgcggccgcatccgggccgtccgcgcggacagctggccgcgcccagcccgaaccgacgcccaggatcgagcgagggcggcgcgcccggggcttggcttagcgtccacgccacctccggctatataagccgccccacacccgctccccctccggcattccattccgccaccgcaccaccaccaccaccaaaccctagcgagcgagcgagggagagagagaccgccccgccgcgacgatggagagatcccgcgggctgctgctggtggcggggctgctggcggcgctgctgccggcggcggcggcgcagccgggggcgccgtgcgagcccgcgctgctggcgacgcaggtggcgctcttctgcgcgcccgacatgccgacggcccagtgctgcgagcccgtcgtcgccgccgtcgacctcggcggcggggtgccctgcctctgccgcgtcgccgccgagccgcagctcgtcatggcgggcctcaacgccacccacctcctcacgctctacagctcctgcggcggcctccgccccggcggcgcccacctcgccgccgcctgcgaaggtacgttgtccgcctcctcccctccctccctccctccctctctctctacgtgctcgctttcctgcttacctagtagtacgtagtttcccatgccttcttgactcgctagaagtgctccggtttgggtctgttaatttcctcgctgtactaccggatctgtcgtcggcacggcgcgcggcgtcgggtcctcgccttctcccgtggcgaccgacctgcgcagcgcgcgcgcggcctagctagcttcataccgctgtacctcgacatacacggagcgatctatggtctactctgagtatttcctcatcgtagaacgcatgcgccgctcgcgattgtttcgtcgattctagatccgtgcttgttcccgcgagttagtatgcatctgcgtgcatatgccgtacgcacgcagatgcagagtctgttgctcgagttatctactgtcgttcgctcgaccatatttgcctgttaatttcctgttcatcgtgcatgcagtagtagtagccatgtccacgccttcttgttttgaggcgatcatcgtcgagatccatggctttgctttctgcactatcttctgccttgttttgttctccgcagtacgtacgtcttgcttggtcaaaactgaaaaacgctttgctgtttgtttgatcggcaagagctggccgtgcttttggcaccgcagtgcgtcgcctctgccgcttttgcgaaacatttccatgttgatcctctggcggaactactttttcgcgtgcggtttgcgtggccttcctctctcgtgaaaagaggtcgggtcaaaccaaatggatcgcctcttggcagagcagcggcagcagatagctggccgtctcgcagctttggcagaaccggtctgtggccatctgtcgccgcctgccaccgtttccctgatgtttgtttctctctcgcctgccactgtttcttttcttgttgcgcacgtacgtcgtcacctcctcctacttttttgccagttttgtttacttttgatgaaatatacggatgaatcggctggtgattaactttggctgctgctgttaattactgtggattttggatgcaggacccgctcccccggccgccgtcgtcagcagccccccgcccccgcctccaccgtccgccgcacctcgccgcaagcagccagcgcgtaagaacctctccctctccctctctctctccctctcgcctgcatctcgctatgtttatccatgtccatatgttgatcagccttgtttagttactaacatgtgcaccggatcgggttctcgcagacgacgcaccaccgccgccaccgccgtcgagcgagaagccgtcgtccccgccgccgtcccaggaccacgacggcgccgccccccgcgccaaggccgcgcccgcccaggcggccacctccacgctcgcgcccgccgccgccgccaccgccccgccgccccaggcgccgcactccgccgcgcccacggcgccgtccaaggcggccttcttcttcgtcgccacggccatgctcggcctctacatcatcctctgagtcgcgcgccgaccccgcgagagaccgtggtccgtccagtcgcagtagagtagagcgctcgtcgtctcgttccgtttcgtgcctgtcgccgttcgaggttcgtttctgcgtgcagtccggtcgaagaagccggtgggttttgagtactagtggtagtagtagcagcagctatcgtttctgtccgctcgtacgtgtttgcgtggtcgcggagaacaattaattgggtgtttgcgagtcctctggttaagatgaaccactgatgctatgtgatcgatcgatcggtatgatctgaatggaaatggatcaagttttgcgttctgctgatgatgtgatccatttggatctgtgtggggcaacagtttcgcttgcttttgctctgcgatgaacgaatgcttcttgcatgcatcttgtctttgcttaatttgaactgtagaacggatgcagtactgatttctgcttatgatgtgacgattcgtcgtacgcatatcatctcttcaaatttgtgtagcagctgtttgtagcttccattctgctatggacgaatgcctgtttttcacggagaaccgcgcgcggggaccgatgcggctttgtgttgccatgttgttttccacgccaggacaaaatagatggtgcggttttgatccccaatcccaccatcaccatgttccggagagccacatggaactcacgtcaagcggtcactttttgcagaatcactcttaccattttacccttttgttgaaacctctctcctcatccccaaaagttgatgcaacagtgctatgcgcgcccacccatgctttttcatatgattgtaaaatttggatcgattttatcttttgaaccctaagtccggtttacaatctgtttgcatgtttatgttccttgcggcgaggaccattaaacaagactactattggatatatttcgacaggctttgaaatccgaattc

SEQ ID NO: 7 - DNA, 4335 bp, Artificial Sequence
  synthetic DNA of Ms1
aagcttaaaccatttagttacaaatatcgatgcacaccttcggtggggcgttgtgaaaaagcatgttttttgggtcgacaagccccttttgcaacgtatcctcttctaatcctattcagatcattaacatcataagctgcaattgacatgctcttctgaggatcaggttcatgcaattaaacatcataaactgcatctttgatgtcatccttttcctatattttttccagattattggcttgcttcgttttcaatatcaggttctatgattcgacttctgttgttgccagtaataatttgtagttgctgcggaatatgaactcaaggagagctgatggtgctatgaagttgatttgatgggaggttgttctacacctgcacttgctgctcgacttaaatacatgccttggatttcttcccagctctagtacataatatttttcaaattaatgttccacgacataaaatttaaatccacaaacatatttttagtacatgaacaattttctaatatagggcaaacatttttcatatacaaaccgatcattttaatatatggtgaaaatcagtgtaatatatgctgaaatgttttcaaatacatattgaacatatttataataaatggtgaacattttttttaataattgatgaccatttttaaaatgcatattgaacattttataatatacactgtacagttttataataatcgacgaacatcttttggagttctgaacatttttttcaaaaacacaagccattttccaggaagaatacaaatgcaaaagaaatgagatatccaaaaagcaaaaaagaaaaacaaaacaaaacagagaaacctacaggaaaatccaaacagaaaaggcaaagaaagaacccgaactgggccaggcaatgtttccaacggcctcgctcttcctgaacaagaaggccagtcagcccatgggctgctcccagtactcgggccccgctgtggcagcacgccatgtaatagttttcgcgggaatccaacgccgaaatcgcccgcagcgggaacccgacgtcggtctggtgcgttctggcgccttccagaactctccacaggctcccgcagccgtccgatcagatcagcacgaagcacgaacattggcgcgcggcgatattttctttcctcgcccgacgacggccgcactgcatttcattttgaatttcaaaattcggaaacggaatagctttctcgcatcccgaggcgaggcggttacgggcgccagaggggccaccccacccacccacccccgccctcacgtgccccgcgcggccgaatccgggccgtccgcgcggacagctggccgcgcccagcccgaaccgacgcccaggatcgagcgagggcggcgcgcccggggcttggcttagcgtccacgccacctccggctatataagccgccccacacccgctccccctccggcattccattccgccaccgcaccaccaccaccaccaaaccctagcgagcgagcgagggagagagagaccgccccgccgcgacgatggagagatcccgcgggctgctgctggtggcggggctgctggcggcgctgctgccggcggcggcggcgcagccgggggcgccgtgcgagcccgcgctgctggcgacgcaggtggcgctcttctgcgcgcccgacatgccgacggcccagtgctgcgagcccgtcgtcgccgccgtcgacctcggcggcggggtgccctgcctctgccgcgtcgccgccgagccgcagctcgtcatggcgggcctcaacgccacccacctcctcacgctctacagctcctgcggcggcctccgccccggcggcgcccacctcgccgccgcctgcgaaggtacgttgtccgcctcctcccctccctccctccctccctctctctctacgtgctcgctttcctgcttacctagtagtacgtagtttcccatgccttcttgactcgctagaagtgctccggtttgggtctgttaatttcctcgctgtactaccggatctgtcgtcggcacggcgcgcggcgtcgggtcctcgccttctcccgtggcgaccgacctgcgcagcgcgcgcgcggcctagctagcttcataccgctgtacctcgacatacacggagcgatctatggtctactctgagtatttcctcatcgtagaacgcatgcgccgctcgcgattgtttcgtcgattctagatccgtgcttgttcccgcgagttagtatgcatctgcgtgcatatgccgtacgcacgcagatgcagagtctgttgctcgagttatctactgtcgttcgctcgaccatatttgcctgttaatttcctgttcatcgtgcatgcagtagtagtagccatgtccacgccttcttgttttgaggcgatcatcgtcgagatccatggctttgctttctgcactatcttctgccttgttttgttctccgcagtacgtacgtcttgcttggtcaaaactgaaaaacgctttgctgtttgtttgatcggcaagagctggccgtgcttttggcaccgcagtgcgtcgcctctgccgcttttgcgaaacatttccatgttgatcctctggcggaactactttttcgcgtgcggtttgcgtggccttcctctctcgtgaaaagaggtcgggtcaaaccaaatggatcgcctcttggcagagcagcggcagcagatagctggccgtctcgcagctttggcagaaccggtctgtggccatctgtcgccgcctgccaccgtttccctgatgtttgtttctctctcgcctgccactgtttcttttcttgttgcgcacgtacgtcgtcacctcctcctacttttttgccagttttgtttacttttgatgaaatatacggatgaatcggctggtgattaactttggctgctgctgttaattactgtggattttggatgcaggacccgctcccccggccgccgtcgtcagcagccccccgcccccgcctccaccgtccgccgcacctcgccgcaagcagccagcgcgtaagaacctctccctctccctctctctctccctctcgcctgcatctcgctatgtttatccatgtccatatgttgatcagccttgtttagttactaacatgtgcaccggatcgggttctcgcagacgacgcaccaccgccgccaccgccgtcgagcgagaagccgtcgtccccgccgccgtcccaggaccacgacggcgccgccccccgcgccaaggccgcgcccgcccaggcggccacctccacgctcgcgcccgccgccgccgccaccgccccgccgccccaggcgccgcactccgccgcgcccacggcgccgtccaaggcggccttcttcttcgtcgccacggccatgctcggcctctacatcatcctctgagtcgcgcgccgaccccgcgagagaccgtggtccgtccagtcgcagtagagtagagcgctcgtcgtctcgttccgtttcgtgcctgtcgccgttcgaggttcgtttctgcgtgcagtccggtcgaagaagccggtgggttttgagtactagtggtagtagtagcagcagctatcgtttctgtccgctcgtacgtgtttgcgtggtcgcggagaacaattaattgggtgtttgcgagtcctctggttaagatgaaccactgatgctatgtgatcgatcgatcggtatgatctgaatggaaatggatcaagttttgcgttctgctgatgatgtgatccatttggatctgtgtggggcaacagtttcgcttgcttttgctctgcgatgaacgaatgcttcttgcatgcatcttgtctttgcttaatttgaactgtagaacggatgcagtactgatttctgcttatgatgtgacgattcgtcgtacgcatatcatctcttcaaatttgtgtagcagctgtttgtagcttccattctgctatggacgaatgcctgtttttcacggagaaccgcgcgcggggaccgatgcggctttgtgttgccatgttgttttccacgccaggacaaaatagatggtgcggttttgatccccaatcccaccatcaccatgttccggagagccacatggaactcacgtcaagcggtcactttttgcagaatcactcttaccattttacccttttgttgaaacctctctcctcatccccaaaagttgatgcaacagtgctatgcgcgcccacccatgctttttcatatgattgtaaaatttggatcgattttatcttttgaaccctaagtccggtttacaatctgtttgcatgtttatgttccttgcggcgaggaccattaaacaagactactattggatatatttcgacaggctttgaaatccgaattc

SEQ ID NO: 8 - DNA, 4504 bp, Oryza sativa
gaacagtgcactggttgggataacaagaagttagaaattgggcatatatatagaagggtaagacacctctaatggatagggtggacaatccatcaaagatgactattttggcacctctgaggccgtgacaagttgcctatcttcgcacccttcacaagtgactccctacttgtgatgggtcgtgagatgtgagccggtgatctttctcagatgtaaatttcggcctctcacaagtgactccttatctgtgataggtcttgccctcacagcctcatctgtaacggcctctaattcaatccgttacagattaaatcattcatgacaagacactttgacccatcataggtgggttgttaatgttgaaccgaggtagcgtggtggtggcttctttgattgttgagcgggttgtgttcttcatcacttggtaggaagtaggaacccaagaaggttagaagcccacaactattatatcgtcggcctcattggtaaatgggctagaagcctagaggcaatctgattcaatagtgtcggaaatttgtggatgggccagagacgttgcgtcgtcttcgactcttcgagtgcctggcctacggatctgcacgaatcttagagcaagtagaaaatcgcatatcgtcgtgtagagcgcagcacaaattcgagttgcttttccctttttcgcagccaaatcttacctgctcacgtgccgtgctgcccggtgtgcagagcccacgcgccacggcgccagtgtactacaccgaatcggcaccatccatcgccacagctggccggtcccccctaagacggacgctccggatcaatccacgttggcatggcttccccgcatcgccttctccgcgcccccgcctatataatggcgctctcgcttctcttccccatttcgtcttccccttctctagagccttcctctcacagagcacacacaaaaccctagagtaggaagcgagcgagagagagagagagagagagagagaccacacccatggagcgctcccacctcgccgtcctgctcggcctcctcgccttcgccgccggggtcccggccgcagcggcggccaccgccgtggagggagcgcaggcggccacggcggaggcgtcgtgcgagccctccatcctcgccacccaggtctcgctcttctgcgcgcccgacatgcccaccgcgcagtgctgcgagccggtggtggcctccgtcgacctcggcggcggcgtaccctgcctctgccgcgtcgccgccgagccgcagctcatcatctccggcctcaacgccacccacctcctcacgctgtacgccgcctgcggaggcctccgccctggaggcgctcgcctcgccgccgcctgtgaaggtacgtacatgcataacctcctcctcctcctcctcctctctctctctctctctctctctctctctctctctctctctctctctctctctctctctctctctctctctctctctctctctctctctctctctctctctctctctctcggttggggttgctgccttgcgtttttggttggtttttcgtgggttgggcgagatccttcgagttgcttgtgttttgtggtatgctaggcttcgaacgagttgccggcgttgctgtgtcgaccaactctcgtatgcttatctttcagcacatgagttttggcctcgtttttactcggttgttgtatgctacttctgagatttgagttcatccactgctaaactgacatcatagatgaagaatagcagcggcgtttggtcgattttgattcctttctctggatgttcgagctgatcttgtggttattgctcgaagcctcgaaacgcttgcgcacatgcaagatccagcaacgtatagatctatagtggtgttgtgcttttattcggatttgtggttcagtgtttacgtgcgaagtcacgcgttcgatgtttccgcttgagctccatatctatagcacaaatcaatcatgtgcgttgcgcgagttcaagctcgagagaaaagaaaagcatcaaggccacggggggtttttgggccaggtcgtgattctcccttgaactccgaatataccgagtttattatcttttgagcggatttggtgttgaactggcaggactcaaaacccacccgtgggacgatcgttttcttttcctttcgctttgtgttctctgtctcctttccgtgaaatctctgcgtttcccttctggtgcttgttatagatgattctggatcgagccgtgtatgctcgtgcagtggtacgacttggcgatgaacgtgcttgcggagctagtcgcagttcatctttcttttttttttccctcgtttcttttctcggcgtttcattctctacacctcttctactcgccatgcatgttcatctctctccgtgttggtcctcatttggagccgattcgaaccgggcagcacagtgctttttttctgtttcgttttggaggtttccactttcgtgaaaaggaaagggtcaaatcgaatcgccccctgaaccatcctttgcagagcttttttggacgtttccgcctttcgtcagagaccatctgcactgcgcgtttctccccaactcgatcgattttgcagcttttaatcactttttagaaaaagtttttaatcactcgtcatcgatgtgatctcttgctctaattgcatcttctccgtaggattagcacttccatgcttcttgttttgtctgttcaattagccaagaaacgagtcagtataccttcaagatgcatgcagatttaaaatcggcactgctctttatcttgttcttgtttttgcaagttttggttggttcaaaacttatctcttctgcagcattgcctgctgtgtacagaaagttggcaggggcatcgtgcagcttttttgcctgctgtgtgtaacgttttctttccgtacgttgcgttccgtttcacgtcgcttacctctgtttcttggggcgcaagttatggcagtacagccgttgtttccacgttggaaggacggttttgccccttcgcttccagaagcttccagagatttttcgagtttttctaatgtgtttgttattgctgtaactcgttctaacgtgcaggtcccgccccaccggcctccatcgtcactgccccgccgcccccggttgcttttcgccgcaagccgccggcacgtaaggctgattgattccccttcatccactgattgttaatgcgcgtgtaatctttgtgattactaacttgctgctggatgctttgcaggcgaggcacctcccccaccgccggcggccgagaagctctccccgccgcctcagcagcacgacgactccgaccacaacaagcgcgtcggcccactcccgagaggctctcctcccccgtatgcccagtccgtcccggtcggccccgccgccgctcccccgccaccacgctccggcgcctcctcgtcgctccaggcgcccctcgccgccaccaccaccatcgttgccatcaccctcatcgccgccgcccagtactgaggacacgccgccgccggcgcccgctccccagagccatgattcgttcgcagtatttttcatcctgttcttttgcttctctctctggctacccatgtatatgagtttggaagacgatgatttgatctagtagcgcgttaccaagtttgcctagattcgagtagtagctgtggtactatgctgatgtctctttgatcgcgtcgtctctagagcgtccgccgtttttgatcgatcactagcatggccgatgtgagtccagcatgaaaagtggtcgaggagaacattgttgctaagttttttttttgctttctatctccagtagctgaacaagtatgtcaactgaatgctgcaatgaagtgaatggatgcagtcttaaatttagcctttctgttgccaacttcttcctctgttctgtacggttcagatgctgcttgttctgtttatgcgatggtgttgcattgttgtgatgtgtgaagtgcgcccaattctgggtgaactctgcagtattggcaagctctgatcgatacataaagaactgaaatgtgccggcttctccgcctcccgttgcatgctcttgtgcgcgagctgcacagcgcaaccgcgccctcctctgcacatccatcgacacaaagtctcaagttgttgcgcgtgtgctctaccaggcaccgtggctcctgcgggcgtgcacgggtcacattcacatcgcacccaagttgcggacgtttcagctgagcacctaccatccgcaatgtttgcccacagcttgctcgatgaaatgactggttcatgtcaaaaggtaaaaactgacattctcacgcggtaaattcccctaagcttcatagaccaccgcactgtcatccactcgacctgccacgacacccgccaccgcagaacgcgacaccctgtgcccacggccacctaccctggcacgcaccgagccgaagccggataagcacccgagttgatccccatgagacgtggcgactcggctgccctctgccac

SEQ ID NO: 9 - DNA, 687 bp, Artificial Sequence
  cDNA of OsMs1
atggagcgctcccacctcgccgtcctgctcggcctcctcgccttcgccgccggggtcccggccgcagcggcggccaccgccgtggagggagcgcaggcggccacggcggaggcgtcgtgcgagccctccatcctcgccacccaggtctcgctcttctgcgcgcccgacatgcccaccgcgcagtgctgcgagccggtggtggcctccgtcgacctcggcggcggcgtaccctgcctctgccgcgtcgccgccgagccgcagctcatcatctccggcctcaacgccacccacctcctcacgctgtacgccgcctgcggaggcctccgccctggaggcgctcgcctcgccgccgcctgtgaaggtcccgccccaccggcctccatcgtcactgccccgccgcccccggttgcttttcgccgcaagccgccggcacgcgaggcacctcccccaccgccggcggccgagaagctctccccgccgcctcagcagcacgacgactccgaccacaacaagcgcgtcggcccactcccgagaggctctcctcccccgtatgcccagtccgtcccggtcggccccgccgccgctcccccgccaccacgctccggcgcctcctcgtcgctccaggcgcccctcgccgccaccaccaccatcgttgccatcaccctcatcgccgccgcccagtactga

SEQ ID NO: 10 - DNA, 5291 bp, Brachypodium distachyon
cccttaaaagggggtaatgatggctcatattgaggaattgacatgcaccccttaaaggaggtaatgatggctcatattgatttgaggaaactccttccataaggacatctccaacaagacacagtcagcggtactataaagcacggcacctggatcagttctcgtcgagggtgcagacgacgattgcagtgaatatgatgactatcgcggcgacgaggagggggggcagtggggacggctgaggtgcatcctctgccaaattaaagcacgcgcgcgtgccacgcgagtcagatcaaggacacgcaaaacagataacatattaacaggaagcaacgcatagatttttagaatcgagtaaaagaatagcagcagcattttttttagcgaaatagtagcagcaattagatcaagcgaaatgtaaaggttgttcacataccaacaagggcggcggtgtggggcgggacattgacctccggggcctcctccagggcctgcggcgcctgctgggcctcgacaaatgcagtcaggctgcaagatatgagggtaaaaaaacagatgtacagtccggtcaagaaaaacaacaaacatgcagactacttagatctgccaagactaaattacctaacgattccaagtccagtgatggttgcatcgcgatgaatttcagccatgctgcgtgcccgcctggttaccggacgcgcgggaaggggagcaagcccaatcagagcgggtgcagccgggcggcgtgtgttattgcgataatactcgacggtatgcttccaccgcaggtacagtctcaggaaggcatccgattgacccaccagatcatctatcaccaaggtagccattctgccacccatctaaacacaaactgagagtaagaaagcagtttgaccgcgattgtttatcacaaaaggcaacacaaaaaaactgctagcttcgtgtcagaaaatcaacatgcatggtgcgcgacagtacaacagaaacatggggagacatagcagaaacgtccaaaccaaaaatccaaaaaaagaaggagatgcactgcgtaagaaaacagcacgggaagcgctcttcaccgtgtgagactgcacaagtccaagagacgacaatagcagaaaagaactgcagaaaggagagctgctttcgggggtcaaagtactagcacggcttcgatcaatcggtcgattaaatccctcgtgccaccgagatcctcacagtgctcgaggggacactctaagtcggctttgtcacatccaacccaaacaacacgctcttgtctaaggtgctcaacaaaggtgatgtgttcgcacgcaggcacagtggaacaacaaactagcgtcgatcgaccacgtccctcccccagaaaagtgctcccaacatgatcgcatcgaagtaatcgtagagatagatcttacagaataaaaaataaacccaaaccaaaggaggagttctgcactactagatccgaaccaaagccaggaaatagcaaactaaacacaaaagatatcgatgaaatcatacatcgtccaaacgtttcggattacaccttctggtcgcaactctcgtgctcaccgcgcagacagatcttctgtacgtaccttggctccagcccgaggagagcgagcactccaggaaacggcggtctcgagcgagcagtctaggaaatggcggtcgcgatggaaaagccttcaagagatatcgggtgatgccccctatttctagagctctggcctttacagttcaccacttcaccctgcgccatcccgattcccagtacctatgacgagcgacgaccctcacgtgcctggccagcatcacgggagagaatcttgctcagcatctcaaccgcccaaacagacagctgtccggtcccacccaaatggacgcacaggatcgatcgggccgccggtggcctgtccttggctaacccttcacgcctcttcgtcccctccgcctatataatcccaccccgctccgcttcttcccccaccgcgctctcttcctctggactcacaccaactcgcctagccctagcggtaggaagcgaaagcgagagatcccacccatggagagatcccaccacctcctcctcgtgctcggcctcctcgccgcgctgctcccggcggccgcggctaccttcgggacgacgcagccggagcctggggccccatgcgagcccaccctcctcgccacccaggtctcgctcttctgcgcgccggacatgccgaccgcgcagtgctgcgagcctgtggtggcctccgtcgacctcgggggtggcgtcccctgcctctgccgtgtcgccgccgagccgcagctcgtcatggccggcctcaacgccacccacctcctcacgctctacacctcctgcggtggactccgccccggaggcgcccacctcgccgccgcctgtgaaggtacgcgacgcctgcgtctctctctctctctgcgtctctctctgcgtctctcccatgacgagcaactcgcgatacgccttactgccttattttttttgaagatatgtgtctgcttggtccactgtatttgggttcttctttcgagaagttcatccgtaggcatctataatccgacgagttcggatgagatcaaacagtgacacgcgcgacaccaacgttttcaacgatctcttgctgtttggtttgatatttcctgcttcccatgatctattttcaaccttttttgtatggctttcgctccaatctcgtgcagaaccatatttcatcttgggtttatgctgttctgtaagatctagcgccatgcagaggtcatttctgctgttccagaccccctacgtgacatttgctgtttttcctctttgttgccatggccacgggttggtttttacgaaagatactttgatatgtcaagatctgcgagcactttgaaaccccaacgcattttctatgtgttttgtgctgtttgatcgaccgattgatcgaggccgtgctagtactttgacacccgaaagcatctctcctttctgcagtatcttttctgttcttgtcgtctcttgggcttgtgcagtttaccatggtgaagagcgcttcatacacgatctgccgcgaggccagagcaaaagcttcccgtgctttttcttgcacagtgcatctccttcttttttgcctttttcgtttggacgtttctgcttcgtctccccatgtttctgttgtactgtcgcgcaccatgcatgttgattttctgatacgaagctagtactgctctgcagtttttgtgtagccttcctctttcgtgataaagaacgtggtcaaactgctctctgactctgttcgtctaaatctttttctcgcaggaaaattttcgttgcagatctcctttaccctcgtcctccgcatctgtttgctttacctgctgtagttgcgttcttcgtttgaatcaaattcttgtttccttcttttatcccatcgctcgtttagttaccttttctttttattgaactttagttcattggtgtagtaggcagtagtatgctttgcgttgtttgcggagtagcaattgaattgctctccggtctctgcagagcggcccgctgaacagatagctggctgcagcagctttaccagaatcggtcggttacgaacttacgattatacccttcgtcttgctttcatttactggtagcctgctagtcttttcttgttgcgcacgtaatcgtacccagtactgtacgcttagataaaatagacgggtctggccttaaattatttcgttgcgttttcgaattttgaattccggaagttaactttattttgtgctctgtttggacgcatgtgcaggtccagctcctcccgccgccgtcgtcagtgcccctcccccctccgccgcacctcgccgcaagcagccagcacgtacgaacaaccttttacacttcgcttgatctaattgctgctgctatactctcttactcgattctaaatctatgttttgctcattattaatatgttgatctgactcgtgtggcacgcgcgcgtgctttgatttcgcagacgaggcacctccgcctccgccgtcgactgagaagccgtccccgccgcctcagcaggacaacgtcaccgcccacggcaaggcaatccccacccatgcggccacatccccgctcgcgccggctgcttccatgatccacatgtccccaccgcccgcatgcaatccatgctccggctccgccgcttcctcagccgaggggcccctcctcatcgccgcgctcctcctcgtcatcaccgccatcatcgtcggcaccctcgacgataagtgatccaggagccgtccgccccctccgactcaccaacgtccgactatgatccagttgcagtagtggtcttgttctgtttcatgtttctcgccatttggttccgagatttctatatcgtgcctagtcgtagctgtagcagtcagtatgttcatgtgtccacaagatgtggtcgagtataacattgggtttcatgattcctctagcagatgaaacactatgtgatgtgatctgaatggatgcagttttgctaccttttctgctgctatgatatgcttatccatatgtttatctttcattcccttaatttgtgcggtttagcgttgtgttgccatgaatgcctcttgctctgctttgcgggttgcattttgtcttcgttctgctgtatatttgattctgaatttgcatgctgtgagtactaagtactgactacaatctctggatggttttgaaatttgaatgatgttataaaggagagctagctggggaattgcctcacctctaaactccaaaacacagagcagaagttggcctcaagatccaacttggtcactttgcatgtcggagcattgtagcaattctgcaataaacggagtagttctgttagcatgttgtttttacactgtcagtacaagtagaggtcgatgattaattatattccggttgtttgctgctggcttcccagttccctccaggtaggaaggaaccgtatccgggtagtagccagtagtagccaggaagctactagcagaacagtcttctggtgctctttttttggagtaacgtcttctcgcgatctttttcgagtaattcaaatccgggtataccgagccttgtatcagtgagagccgatagtcttaattatctccagcacaggcacaggaacaaccacgtttgtttttcagaatgcacagcaacattttttttaagagcatggcacagctactttttttttttttaaggaaacatggcacagctacatttttttttagaggaacatggcaca

SEQ ID NO: 11 - DNA, 687 bp, Artificial Sequence
  cDNA of BdMs1
atggagagatcccaccacctcctcctcgtgctcggcctcctcgccgcgctgctcccggcggccgcggctaccttcgggacgacgcagccggagcctggggccccatgcgagcccaccctcctcgccacccaggtctcgctcttctgcgcgccggacatgccgaccgcgcagtgctgcgagcctgtggtggcctccgtcgacctcgggggtggcgtcccctgcctctgccgtgtcgccgccgagccgcagctcgtcatggccggcctcaacgccacccacctcctcacgctctacacctcctgcggtggactccgccccggaggcgcccacctcgccgccgcctgtgaaggtccagctcctcccgccgccgtcgtcagtgcccctcccccctccgccgcacctcgccgcaagcagccagcacacgaggcacctccgcctccgccgtcgactgagaagccgtccccgccgcctcagcaggacaacgtcaccgcccacggcaaggcaatccccacccatgcggccacatccccgctcgcgccggctgcttccatgatccacatgtccccaccgcccgcatgcaatccatgctccggctccgccgcttcctcagccgaggggcccctcctcatcgccgcgctcctcctcgtcatcaccgccatcatcgtcggcaccctcgacgataagtga

SEQ ID NO: 12 - DNA, 1707 bp, Artificial Sequence
  cDNA of TpMYC4E
atgcgggaaatagctactcagcggtgtggtaatcgatcaatggcgctatcagctcctcccagtcaggaacagccgtcggggaagcaattcggctaccagctcgctgctgctgtgaggagcatcaactggacttatggcatattttggtccatttccgccagcccgcgcccaggccactcctcagttctggcgtggaaggatgggttctacaacggcgagataaagactagaaagattaccggctcgaccactacggagcttacagcggacgagcgcgtcatgcacagaagcaagcaactgagggagctctacgaatcgctcttgcccggcaactccaacaaccgggcaaggcgaccaaccgcctcactgtcaccggaggatctcggggacggcgagtggtattacaccataagcatgacttacaccttccaccctaatcaagggttgccaggcaaaagctttgcgagcaatcaacatgtttggctgtacaacgctcaatacgcaaacaccagagttttcccccgcgcgctcttagcaaagacaatcgtttgcattcccttcatgggcggtgtgcttgagctcggaacgtcggatcaggtgttggaggacccgagcatggtgaagcggatcagcacgtctttctgggagctgcacttgccgtcatccttggagtcgaaggatccgagctccagcacatcagcaaacgataccagggaggccaccgacatcatcttgttcgaggatttcgaccacaacgacacagttgagggggtgatctctgagcaaagggaggtccagtgcccgtccaacgtcaatctggagcgcctcacaaagcagatggacgagttccacagccttctcggtggactggacgtgcatcctctcgaagacagatggatcatggacgagccctttgagtttacgttttccccagaagtggcgccggctatggatatgccgagcaccgacgatgtcatcgtcactttaagtaggtccgaaggctctcgtccatcctgcttcacagcgtggaagggatcatccgagtcgaaatacgtggctggccaggtcgttggggagtcacagaagttgctgaataaagttgtggctggtggtgcatgggcgagcaattatggcggtcgcaccatggtgagagctcagggaattaacagcaacacccatgtcatgacagagagaagacgccgggagaaactcaacgagatgttcctggttctcaagtcactggtcccgtccattcacaaggtagacaaagcatccatcctcacagaaacgataggttatcttagagaactgaagcaaagggtagatcagctagaatccagccggtcaccgtctcacccaaaagaaacaacaggaccgagcagaagccatgtcgtcggcgctaggaagaagatagtctcggccggatccaagaggaaggcgccagggctggagagcccgagcaatgtcgtgaacgtgacgatgctggacaaggtggtgctgttggaggtgcagtgcccgtggaaggagctgctgatgacacaagtgtttgacgccatcaagagcctctgtctggacgttgtctccgtgcaggcatccacatcaggtggccgtcttgacctcaagatacgagctaatcagcagcttgcggtcggttctgctatggtggcacctggggcaatcaccgaaacacttcagaaagctatatag

SEQ ID NO: 13 - protein, 568 aa, Thinopyrum ponticum
MREIATQRCGNRSMALSAPPSQEQPSGKQFGYQLAAAVRSINWTYGIFWSISASPRPGHSSVLAWKDGFYNGEIKTRKITGSTTTELTADERVMHRSKQLRELYESLLPGNSNNRARRPTASLSPEDLGDGEWYYTISMTYTFHPNQGLPGKSFASNQHVWLYNAQYANTRVFPRALLAKTIVCIPFMGGVLELGTSDQVLEDPSMVKRISTSFWELHLPSSLESKDPSSSTSANDTREATDIILFEDFDHNDTVEGVISEQREVQCPSNVNLERLTKQMDEFHSLLGGLDVHPLEDRWIMDEPFEFTFSPEVAPAMDMPSTDDVIVTLSRSEGSRPSCFTAWKGSSESKYVAGQVVGESQKLLNKVVAGGAWASNYGGRTMVRAQGINSNTHVMTERRRREKLNEMFLVLKSLVPSIHKVDKASILTETIGYLRELKQRVDQLESSRSPSHPKETTGPSRSHVVGARKKIVSAGSKRKAPGLESPSNVVNVTMLDKVVLLEVQCPWKELLMTQVFDAIKSLCLDVVSVQASTSGGRLDLKIRANQQLAVGSAMVAPGAITETLQKAI

SEQ ID NO: 14 - DNA, 669 bp, Artificial Sequence
  cDNA of Ms1 derived from Triticum boeoticum
atggagagatcccgccgcctgctgctggtggcgggcctgctcgccgcgctgctcccggcggcggcggccgccttcgggccgcagccgggggcgccgtgcgagcccacgctgctggcgacgcaggtggcgctcttctgcgcgcccgacatgcccaccgcgcagtgctgcgagcccgtcgtcgccgccgtcgacctcggcggcggggtcccctgcctctgccgcgtcgccgcggagccgcagctcgtcatggcgggcctcaacgccacccacctcctcacgctctacagctcctgcggcggcctccgtcccggcggcgcccacctcgccgccgcctgcgaaggacccgctcccccggccgccgtcgtcagcagccccccgcccccgccaccgtcgaccgcacctcgccgcaagcagccagcgcacgacgcaccaccgccgccgccgccgtccagcgacaagccgtcgtccccgccgccgtcccaggagcacgacggcgccgccccccacgccaaggccgcccccgcccaggcggctacctccccgctcgcgcccgctgctgccatcgccccgccgccccaggcgccacactccgccgcggcgacctcgtcgtccaaggcggccttcttcttcgtcgccacggccatgatcggcctctacctcatcctctga

SEQ ID NO: 15 - protein, 222 aa, Triticum boeoticum
MERSRRLLLVAGLLAALLPAAAAAFGPQPGAPCEPTLLATQVALFCAPDMPTAQCCEPVVAAVDLGGGVPCLCRVAAEPQLVMAGLNATHLLTLYSSCGGLRPGGAHLAAACEGPAPPAAVVSSPPPPPPSTAPRRKQPAHDAPPPPPPSSDKPSSPPPSQEHDGAAPHAKAAPAQAATSPLAPAAAIAPPPQAPHSAAATSSSKAAFFFVATAMIGLYLIL

SEQ ID NO: 16 - DNA, 19 bp, Artificial Sequence
  primer 5565329F
tgcagtgatcccgatgccg

SEQ ID NO: 17 - DNA, 17 bp, Artificial Sequence
  primer 5565329R
ctcggtgcgatgtgtgg

SEQ ID NO: 18 - DNA, 23 bp, Artificial Sequence
  primer 5570804F
tgcaggattttccactgattaac

SEQ ID NO: 19 - DNA, 18 bp, Artificial Sequence
  primer 5570804R
cggaggtggtacgcggtg

SEQ ID NO: 20 - DNA, 26 bp, Artificial Sequence
  primer 5564956F
tgcagaactaccagaatctttatcgg

SEQ ID NO: 21 - DNA, 24 bp, Artificial Sequence
  primer 5564956R
ctgtgaaaccaagcacccataatc

SEQ ID NO: 22 - DNA, 23 bp, Artificial Sequence
  primer 5008421F
tgcagagcaagagcaacattcaa

SEQ ID NO: 23 - DNA, 23 bp, Artificial Sequence
  primer 5008421R
cggtcaatgtataaaccacgtgc

SEQ ID NO: 24 - DNA, 19 bp, Artificial Sequence
  primer 3573220F
tgcagtcagtcaacgatgg

SEQ ID NO: 25 - DNA, 17 bp, Artificial Sequence
  primer 3573220R
gtctcacgtgcagcgca

SEQ ID NO: 26 - DNA, 22 bp, Artificial Sequence
  primer 5565375F
tgcagtttctatcatgtccacg

SEQ ID NO: 27 - DNA, 21 bp, Artificial Sequence
  primer 5565375R
atctcgggtttatcttcaggg

SEQ ID NO: 28 - DNA, 21 bp, Artificial Sequence
  primer 1861695F
tgcaggtgtgctacttagggc

SEQ ID NO: 29 - DNA, 19 bp, Artificial Sequence
  primer 1861695R
cggaccttgccctgaggag

SEQ ID NO: 30 - DNA, 18 bp, Artificial Sequence
  primer 5571044F
tgcagtggaaagtgcggc

SEQ ID NO: 31 - DNA, 26 bp, Artificial Sequence
  primer 5571044R
cggtagatagaagatgagactttacc

SEQ ID NO: 32 - DNA, 23 bp, Artificial Sequence
  primer 5565269F
tgcaggtggacctcatggactac

SEQ ID NO: 33 - DNA, 20 bp, Artificial Sequence
  primer 5565269R
ctcaggcacaccgcgcagtc

SEQ ID NO: 34 - DNA, 20 bp, Artificial Sequence
  primer 5570850F
tgcaggcggtcctggacagg

SEQ ID NO: 35 - DNA, 18 bp, Artificial Sequence
  primer 5570850R
cggccgccctcaccacac

SEQ ID NO: 36 - DNA, 21 bp, Artificial Sequence
  primer 5565089F
tgcagcattggcaaataacac

SEQ ID NO: 37 - DNA, 22 bp, Artificial Sequence
  primer 5565089R
ggttgcattctctgtgtatcac

SEQ ID NO: 38 - DNA, 17 bp, Artificial Sequence
  primer RfF1
gccgccgcctgcgaagg

SEQ ID NO: 39 - DNA, 17 bp, Artificial Sequence
  primer RfR1
gggggagcgggtcctgc

SEQ ID NO: 40 - DNA, 18 bp, Artificial Sequence
  primer ThMYC4ESpF
ctcccagtcaggaacagc

SEQ ID NO: 41 - DNA, 18 bp, Artificial Sequence
  primer TaMYC4SpR
ggtgacagtgaggcggtt

SEQ ID NO: 42 - protein, 228 aa, Oryza sativa
MERSHLAVLLGLLAFAAGVPAAAAATAVEGAQAATAEASCEPSILATQVSLFCAPDMPTAQCCEPVVASVDLGGGVPCLCRVAAEPQLIISGLNATHLLTLYAACGGLRPGGARLAAACEGPAPPASIVTAPPPPVAFRRKPPAREAPPPPPAAEKLSPPPQQHDDSDHNKRVGPLPRGSPPPYAQSVPVGPAAAPPPPRSGASSSLQAPLAATTTIVAITLIAAAQY

SEQ ID NO: 43 - protein, 228 aa, Brachypodium distachyon
MERSHHLLLVLGLLAALLPAAAATFGTTQPEPGAPCEPTLLATQVSLFCAPDMPTAQCCEPVVASVDLGGGVPCLCRVAAEPQLVMAGLNATHLLTLYTSCGGLRPGGAHLAAACEGPAPPAAVVSAPPPSAAPRRKQPAHEAPPPPPSTEKPSPPPQQDNVTAHGKAIPTHAATSPLAPAASMIHMSPPPACNPCSGSAASSAEGPLLIAALLLVITAIIVGTLDDK

SEQ ID NO: 44 - DNA, 1722 bp, Artificial Sequence
  cDNA
atgcgggaaatagctactcagcggtgtggtaatcgatcaatggcgctatcagctcctcccagtcaggaacagccgtcggggaagcaattcggctaccagctcgctgctgctgtgaggagcatcaactggacttatggcatattttggtccatttccgccagcccgcgcccaggccactcctcagttctggcgtggaaggatgggttctacaacggcgagataaagactagaaagattaccggctcgaccactacggagcttacagcggacgagcgcgtcatgcacagaagcaagcaactgagggagctctacgaatcgctcttgcccggcaactccaacaaccgggcaaggcgaccaaccgcctcactgtcaccggaggatctcggggacggcgagtggtattacaccataagcatgacttacaccttccaccctaatcaagggttgccaggcaaaagctttgcgagcaatcaacatgtttggctgtacaacgctcaatacgcaaacaccagagttttcccccgcgcgctcttagcaaagactgcttctattcagacaatcgtttgcattcccttcatgggcggtgtgcttgagctcggaacgtcggatcaggtgttggaggacccgagcatggtgaagcggatcaacacgtctttctgggagctgcacttgccgtcatccttggagtcgaaggatccgagctccagcacatcagcaaacgataccagggaggccaccgacatcatcttgttcgaggatttcgaccacaacgacacagttgagggggtgatctctgagcaaagggaggtccagtgcacgtccaacgtcaatctggagcgcctcacaaagcagatggacgagttccacagccttctcggtggactggacgtgcatcctctcaaagacagatggatcatggacgagccctttgagtttacgttttccccagaagtggcgccggctatggatatgccgagcaccgacgatgtcatcgtcactttaagtaggtccgaaggctctcgtccatcctgcttcacagcgtggaagggatcatccgagtcgaaatacgtggctggccaggtcgttggggagtcacagaagttgctgaataaagttgtggctggtggtgcatgggcgagcaattatggcggtcgcaccatggtgagagctcagggaattaacagcaacacccatgtcatgacagagagaagacgccgggagaaactcaacgagatgttcctggttctcaagtcactggtcccgtccattcacaaggtagacaaagcatccatcctcacagaaacgataggttatcttagagaactgaagcaaagggtagatcagctagaatccagccggtcaccgtctcacccaaaagaaacaacaggaccgagcagaagccatgtcgtcggcgctaggaagaagatagtctcggccggatccaagaggaaggcgccagggctggagagcccgagcaatgtcgtgaacgtgacgatgctggacaaggtggtgctgttggaggtgcagtgcccgtggaaggagctgctgatgacacaagtgtttgacgccatcaagagcctctgtctggacgttgtctccgtgcaggcatccacatcaggtggccgtcttgacctcaagatacgagctaatcagcagcttgcggtcggttctgctatggtggcacctggggcaatcaccgaaacacttcagaaagctatatag

SEQ ID NO: 45 - protein, 573 aa, Thinopyrum ponticum
MREIATQRCGNRSMALSAPPSQEQPSGKQFGYQLAAAVRSINWTYGIFWSISASPRPGHSSVLAWKDGFYNGEIKTRKITGSTTTELTADERVMHRSKQLRELYESLLPGNSNNRARRPTASLSPEDLGDGEWYYTISMTYTFHPNQGLPGKSFASNQHVWLYNAQYANTRVFPRALLAKTASIQTIVCIPFMGGVLELGTSDQVLEDPSMVKRINTSFWELHLPSSLESKDPSSSTSANDTREATDIILFEDFDHNDTVEGVISEQREVQCTSNVNLERLTKQMDEFHSLLGGLDVHPLKDRWIMDEPFEFTFSPEVAPAMDMPSTDDVIVTLSRSEGSRPSCFTAWKGSSESKYVAGQVVGESQKLLNKVVAGGAWASNYGGRTMVRAQGINSNTHVMTERRRREKLNEMFLVLKSLVPSIHKVDKASILTETIGYLRELKQRVDQLESSRSPSHPKETTGPSRSHVVGARKKIVSAGSKRKAPGLESPSNVVNVTMLDKVVLLEVQCPWKELLMTQVFDAIKSLCLDVVSVQASTSGGRLDLKIRANQQLAVGSAMVAPGAITETLQKAI